European Patent Application EP 4 667 493 A2, published December 24, 2025. Title: LAG-3 COMBINATION THERAPY FOR THE TREATMENT OF CANCER. Applicant: BRISTOL-MYERS SQUIBB COMPANY. Application EP 25199065.1, filed July 25, 2019. The sequence listing filed with the application follows.

SEQUENCE LISTING (26 sequences)

SEQ ID NO: 1 - protein, 447 aa, synthetic construct
  source 1..447: note = Heavy Chain Amino Acid Sequence; Anti-LAG-3 mAb (BMS-986016)
QVQLQQWGAGLLKPSETLSLTCAVYGGSFSDYYWNWIRQPPGKGLEWIGEINHRGSTNSNPSLKSRVTLSLDTSKNQFSLKLRSVTAADTAVYYCAFGYSDYEYNWFDPWGQGTLVTVSSASTKGPSVFPLAPCSRSTSESTAALGCLVKDYFPEPVTVSWNSGALTSGVHTFPAVLQSSGLYSLSSVVTVPSSSLGTKTYTCNVDHKPSNTKVDKRVESKYGPPCPPCPAPEFLGGPSVFLFPPKPKDTLMISRTPEVTCVVVDVSQEDPEVQFNWYVDGVEVHNAKTKPREEQFNSTYRVVSVLTVLHQDWLNGKEYKCKVSNKGLPSSIEKTISKAKGQPREPQVYTLPPSQEEMTKNQVSLTCLVKGFYPSDIAVEWESNGQPENNYKTTPPVLDSDGSFFLYSRLTVDKSRWQEGNVFSCSVMHEALHNHYTQKSLSLSLGK

SEQ ID NO: 2 - protein, 214 aa, synthetic construct
  source 1..214: note = Light Chain Amino Acid Sequence; Anti-LAG-3 mAb (BMS-986016)
EIVLTQSPATLSLSPGERATLSCRASQSISSYLAWYQQKPGQAPRLLIYDASNRATGIPARFSGSGSGTDFTLTISSLEPEDFAVYYCQQRSNWPLTFGQGTNLEIKRTVAAPSVFIFPPSDEQLKSGTASVVCLLNNFYPREAKVQWKVDNALQSGNSQESVTEQDSKDSTYSLSSTLTLSKADYEKHKVYACEVTHQGLSSPVTKSFNRGEC

SEQ ID NO: 3 - protein, 120 aa, synthetic construct
  source 1..120: note = Heavy Chain Variable Region (VH) Amino Acid Sequence; Anti-LAG-3 mAb (BMS-986016)
QVQLQQWGAGLLKPSETLSLTCAVYGGSFSDYYWNWIRQPPGKGLEWIGEINHRGSTNSNPSLKSRVTLSLDTSKNQFSLKLRSVTAADTAVYYCAFGYSDYEYNWFDPWGQGTLVTVSS

SEQ ID NO: 4 - DNA, 360 bp, synthetic construct
  source 1..360: mol_type = other DNA; note = Heavy Chain Variable Region (VH) Nucleotide Sequence; Anti-LAG-3 mAb (BMS-986016)
caggtgcagctacagcagtggggcgcaggactgttgaagccttcggagaccctgtccctcacctgcgctgtctatggtgggtccttcagtgattactactggaactggatccgccagcccccagggaaggggctggagtggattggggaaatcaatcatcgtggaagcaccaactccaacccgtccctcaagagtcgagtcaccctatcactagacacgtccaagaaccagttctccctgaagctgaggtctgtgaccgccgcggacacggctgtgtattactgtgcgtttggatatagtgactacgagtacaactggttcgacccctggggccagggaaccctggtcaccgtctcctca

SEQ ID NO: 5 - protein, 107 aa, synthetic construct
  source 1..107: note = Light Chain Variable Region (VL) Amino Acid Sequence; Anti-LAG-3 mAb (BMS-986016)
EIVLTQSPATLSLSPGERATLSCRASQSISSYLAWYQQKPGQAPRLLIYDASNRATGIPARFSGSGSGTDFTLTISSLEPEDFAVYYCQQRSNWPLTFGQGTNLEIK

SEQ ID NO: 6 - DNA, 321 bp, synthetic construct
  source 1..321: mol_type = other DNA; note = Light Chain Variable Region (VL) Nucleotide Sequence; Anti-LAG-3 mAb (BMS-986016)
gaaattgtgttgacacagtctccagccaccctgtctttgtctccaggggaaagagccaccctctcctgcagggccagtcagagtattagcagctacttagcctggtaccaacagaaacctggccaggctcccaggctcctcatctatgatgcatccaacagggccactggcatcccagccaggttcagtggcagtgggtctgggacagacttcactctcaccatcagcagcctagagcctgaagattttgcagtttattactgtcagcagcgtagcaactggcctctcacttttggccaggggaccaacctggagatcaaa

SEQ ID NO: 7 - protein, 5 aa, synthetic construct
  source 1..5: note = Heavy Chain CDR1 Amino Acid Sequence; Anti-LAG-3 mAb (BMS-986016)
DYYWN

SEQ ID NO: 8 - protein, 16 aa, synthetic construct
  source 1..16: note = Heavy Chain CDR2 Amino Acid Sequence; Anti-LAG-3 mAb (BMS-986016)
EINHRGSTNSNPSLKS

SEQ ID NO: 9 - protein, 12 aa, synthetic construct
  source 1..12: note = Heavy Chain CDR3 Amino Acid Sequence; Anti-LAG-3 mAb (BMS-986016)
GYSDYEYNWFDP

SEQ ID NO: 10 - protein, 11 aa, synthetic construct
  source 1..11: note = Light Chain CDR1 Amino Acid Sequence; Anti-LAG-3 mAb (BMS-986016)
RASQSISSYLA

SEQ ID NO: 11 - protein, 7 aa, synthetic construct
  source 1..7: note = Light Chain CDR2 Amino Acid Sequence; Anti-LAG-3 mAb (BMS-986016)
DASNRAT

SEQ ID NO: 12 - protein, 9 aa, synthetic construct
  source 1..9: note = Light Chain CDR3 Amino Acid Sequence; Anti-LAG-3 mAb (BMS-986016)
QQRSNWPLT

SEQ ID NO: 13 - protein, 440 aa, synthetic construct
  source 1..440: note = Heavy Chain Amino Acid Sequence; Anti-PD-1 mAb (BMS936558)
QVQLVESGGGVVQPGRSLRLDCKASGITFSNSGMHWVRQAPGKGLEWVAVIWYDGSKRYYADSVKGRFTISRDNSKNTLFLQMNSLRAEDTAVYYCATNDDYWGQGTLVTVSSASTKGPSVFPLAPCSRSTSESTAALGCLVKDYFPEPVTVSWNSGALTSGVHTFPAVLQSSGLYSLSSVVTVPSSSLGTKTYTCNVDHKPSNTKVDKRVESKYGPPCPPCPAPEFLGGPSVFLFPPKPKDTLMISRTPEVTCVVVDVSQEDPEVQFNWYVDGVEVHNAKTKPREEQFNSTYRVVSVLTVLHQDWLNGKEYKCKVSNKGLPSSIEKTISKAKGQPREPQVYTLPPSQEEMTKNQVSLTCLVKGFYPSDIAVEWESNGQPENNYKTTPPVLDSDGSFFLYSRLTVDKSRWQEGNVFSCSVMHEALHNHYTQKSLSLSLGK

SEQ ID NO: 14 - protein, 213 aa, synthetic construct
  source 1..213: note = Light Chain Amino Acid Sequence; Anti-PD-1 mAb (BMS936558)
EIVLTQSPATLSLSPGERATLSCRASQSVSSYLAWYQQKPGQAPRLLIYDASNRATGIPARFSGSGSGTDFTLTISSLEPEDFAVYYCQQSSNWPRTFGQGTKVEIKRTVAAPSVFIFPPSDEQLKSGTASVVCLLNNFYPREAKVQWKVDNALQSGNSQESVTEQDSKDSTYSLSSTLLSKADYEKHKVYACEVTHQGLSSPVTKSFNRGEC

SEQ ID NO: 15 - protein, 113 aa, synthetic construct [sequence omitted]

SEQ ID NO: 16 - DNA, 339 bp, synthetic construct
  source 1..339: mol_type = other DNA; note = Heavy Chain Variable Region (VH) Nucleotide Sequence; Anti-PD-1 mAb (BMS936558)
caggtgcagctggtggagtctgggggaggcgtggtccagcctgggaggtccctgagactcgactgtaaagcgtctggaatcaccttcagtaactctggcatgcactgggtccgccaggctccaggcaaggggctggagtgggtggcagttatttggtatgatggaagtaaaagatactatgcagactccgtgaagggccgattcaccatctccagagacaattccaagaacacgctgtttctgcaaatgaacagcctgagagccgaggacacggctgtgtattactgtgcgacaaacgacgactactggggccagggaaccctggtcaccgtctcctca

SEQ ID NO: 17 - protein, 107 aa, synthetic construct [sequence omitted]

SEQ ID NO: 18 - DNA, 321 bp, synthetic construct
  source 1..321: mol_type = other DNA; note = Light Chain Variable Region (VL) Nucleotide Sequence; Anti-PD-1 mAb (BMS936558)
gaaattgtgttgacacagtctccagccaccctgtctttgtctccaggggaaagagccaccctctcctgcagggccagtcagagtgttagtagttacttagcctggtaccaacagaaacctggccaggctcccaggctcctcatctatgatgcatccaacagggccactggcatcccagccaggttcagtggcagtgggtctgggacagacttcactctcaccatcagcagcctagagcctgaagattttgcagtttattactgtcagcagagtagcaactggcctcggacgttcggccaagggaccaaggtggaaatcaaa

SEQ ID NO: 19 - protein, 5 aa, synthetic construct
  source 1..5: note = Heavy Chain CDR1 Amino Acid Sequence; Anti-PD-1 mAb (BMS936558)
NSGMH

SEQ ID NO: 20 - protein, 17 aa, synthetic construct
  source 1..17: note = Heavy Chain CDR2 Amino Acid Sequence; Anti-PD-1 mAb (BMS936558)
VIWYDGSKRYYADSVKG

SEQ ID NO: 21 - protein, 4 aa, synthetic construct
  source 1..4: note = Heavy Chain CDR3 Amino Acid Sequence; Anti-PD-1 mAb (BMS936558)
NDDY

SEQ ID NO: 22 - protein, 11 aa, synthetic construct
  source 1..11: note = Light Chain CDR1 Amino Acid Sequence; Anti-PD-1 mAb (BMS936558)
RASQSVSSYLA

SEQ ID NO: 23 - protein, 7 aa, synthetic construct
  source 1..7: note = Light Chain CDR2 Amino Acid Sequence; Anti-PD-1 mAb (BMS936558)
DASNRAT

SEQ ID NO: 24 - protein, 9 aa, synthetic construct
  source 1..9: note = Light Chain CDR3 Amino Acid Sequence; Anti-PD-1 mAb (BMS936558)
QQSSNWPRT

SEQ ID NO: 25 - DNA, 1344 bp, synthetic construct
  source 1..1344: mol_type = other DNA; note = Heavy Chain Nucleotide Sequence; Anti-LAG-3 mAb (BMS-986016)
caggtgcagctacagcagtggggcgcaggactgttgaagccttcggagaccctgtccctcacctgcgctgtctatggtgggtccttcagtgattactactggaactggatccgccagcccccagggaaggggctggagtggattggggaaatcaatcatcgtggaagcaccaactccaacccgtccctcaagagtcgagtcaccctatcactagacacgtccaagaaccagttctccctgaagctgaggtctgtgaccgccgcggacacggctgtgtattactgtgcgtttggatatagtgactacgagtacaactggttcgacccctggggccagggaaccctggtcaccgtctcctcagctagcaccaagggcccatccgtcttccccctggcgccctgctccaggagcacctccgagagcacagccgccctgggctgcctggtcaaggactacttccccgaaccggtgacggtgtcgtggaactcaggcgccctgaccagcggcgtgcacaccttcccggctgtcctacagtcctcaggactctactccctcagcagcgtggtgaccgtgccctccagcagcttgggcacgaagacctacacctgcaacgtagatcacaagcccagcaacaccaaggtggacaagagagttgagtccaaatatggtcccccatgcccaccatgcccagcacctgagttcctggggggaccatcagtcttcctgttccccccaaaacccaaggacactctcatgatctcccggacccctgaggtcacgtgcgtggtggtggacgtgagccaggaagaccccgaggtccagttcaactggtacgtggatggcgtggaggtgcataatgccaagacaaagccgcgggaggagcagttcaacagcacgtaccgtgtggtcagcgtcctcaccgtcctgcaccaggactggctgaacggcaaggagtacaagtgcaaggtctccaacaaaggcctcccgtcctccatcgagaaaaccatctccaaagccaaagggcagccccgagagccacaggtgtacaccctgcccccatcccaggaggagatgaccaagaaccaggtcagcctgacctgcctggtcaaaggcttctaccccagcgacatcgccgtggagtgggagagcaatgggcagccggagaacaactacaagaccacgcctcccgtgctggactccgacggctccttcttcctctacagcaggctaaccgtggacaagagcaggtggcaggaggggaatgtcttctcatgctccgtgatgcatgaggctctgcacaaccactacacacagaagagcctctccctgtctctgggtaaatga

SEQ ID NO: 26 - DNA, 645 bp, synthetic construct
  source 1..645: mol_type = other DNA; note = Light Chain Nucleotide Sequence; Anti-LAG-3 mAb (BMS-986016)
gaaattgtgttgacacagtctccagccaccctgtctttgtctccaggggaaagagccaccctctcctgcagggccagtcagagtattagcagctacttagcctggtaccaacagaaacctggccaggctcccaggctcctcatctatgatgcatccaacagggccactggcatcccagccaggttcagtggcagtgggtctgggacagacttcactctcaccatcagcagcctagagcctgaagattttgcagtttattactgtcagcagcgtagcaactggcctctcacttttggccaggggaccaacctggagatcaaacgtacggtggctgcaccatctgtcttcatcttcccgccatctgatgagcagttgaaatctggaactgcctctgttgtgtgcctgctgaataacttctatcccagagaggccaaagtacagtggaaggtggataacgccctccaatcgggtaactcccaggagagtgtcacagagcaggacagcaaggacagcacctacagcctcagcagcaccctgacgctgagcaaagcagactacgagaaacacaaagtctacgcctgcgaagtcacccatcagggcctgagctcgcccgtcacaaagagcttcaacaggggagagtgttag